European Patent Application EP 4 538 387 A2, published April 16, 2025. Title: PERONOSPORA RESISTANCE IN SPINACIA OLERACEA. Applicant: Rijk Zwaan Zaadteelt en Zaadhandel B.V. Application EP. The sequence listing filed with the application follows.

SEQUENCE LISTING (8 sequences)

SEQ ID NO: 1 - DNA, 79 bp, Spinacia oleracea
  misc_feature 1..79: note = source = /organism="Spinacia oleracea" /mol_type="unassigned DNA"
  source 1..79: mol_type = genomic DNA
gaggtggttatggaggagtacacaacaaggtacacttcacatctccaccacccccttcattccataccgaaaacttgcc

SEQ ID NO: 2 - DNA, 79 bp, Spinacia oleracea
  misc_feature 1..79: note = source = /organism="Spinacia oleracea" /mol_type="unassigned DNA"
  source 1..79: mol_type = genomic DNA
gaggtggttatggaggagtacacaacaaggtaaacttcacatctccaccacccccttcattccataccgaaaacttgcc

SEQ ID NO: 3 - DNA, 100 bp, Spinacia oleracea
  misc_feature 1..100: note = source = /organism="Spinacia oleracea" /mol_type="unassigned DNA"
  source 1..100: mol_type = genomic DNA
gctcagtgtcatctttatgcagaagtatatcatagaattgtcaaaaaatgatccgatctagaccaacctgataaaaaaaatcggaagtggcttgatctcg

SEQ ID NO: 4 - DNA, 104 bp, Spinacia oleracea
  misc_feature 1..104: note = source = /organism="Spinacia oleracea" /mol_type="unassigned DNA"
  source 1..104: mol_type = genomic DNA
gctcagtgtcatctttatgcagaagtatatcatagaattgtcaaaaaatgatccgatcgatctagaccaacctgataaaaaaaatcggaagtggcttgatctcg

SEQ ID NO: 5 - DNA, 119 bp, Spinacia oleracea
  misc_feature 1..119: note = source = /organism="Spinacia oleracea" /mol_type="unassigned DNA"
  source 1..119: mol_type = genomic DNA
gcagcatgattgacaacttggtttaacttttgctgcnananctcttttttctttcttgtatcctcttttaacttccattcaaaaagaattttgtggtttaggagttgtagtggtggggt

SEQ ID NO: 6 - DNA, 119 bp, Spinacia oleracea
  misc_feature 1..119: note = source = /organism="Spinacia oleracea" /mol_type="unassigned DNA"
  source 1..119: mol_type = genomic DNA
gcagcatgattgacaacttggtttaacttttgctgcnananctcttttttctttcttgtatcctcttttaacttccatccaaaaagaattttgtggtttaggagttgtagtggtggggt

SEQ ID NO: 7 - DNA, 143 bp, Spinacia oleracea
  misc_feature 49: note = /note="n = a or t or c or g"
  misc_feature 1..143: note = source = /organism="Spinacia oleracea" /mol_type="unassigned DNA"
  source 1..143: mol_type = genomic DNA
gtcgatctgacaagtttgagatgtataagtttttctagggatcaatttngtatcaaatgagcggtttaatttcaagtcttgtaatcaaataaaagtctgattttgtcaaatctatcaaaatcataaacaaatatcaagagatg

SEQ ID NO: 8 - DNA, 143 bp, Spinacia oleracea
  misc_feature 49: note = /note="n = a or t or c or g"
  misc_feature 1..143: note = source = /organism="Spinacia oleracea" /mol_type="unassigned DNA"
  source 1..143: mol_type = genomic DNA
gtcgatctgacaagtttgagatgtataagtttttctagggatcaatttngtatcaaatgagcggtttaatttcaagtcgtgtaatcaaataaaagtctgattttgtcaaatctatcaaaatcataaacaaatatcaagagatg